European Patent Specification EP 3 796 922 B1, published March 18, 2026. Title: PHARMACEUTICAL COMPOSITIONS FOR THE TREATMENT OF CANCER. Applicant: Seleq. The sequence listing filed with the application follows.

SEQUENCE LISTING (3 sequences)

SEQ ID NO: 1 - protein, 422 aa, Homo sapiens
MAKQLQARRLDGIDYNPWVEFVKLASEHDVVNLGQGFPDFPPPDFAVEAFQHAVSGDFMLNQYTKTFGYPPLTKILASFFGELLGQEIDPLRNVLVTVGGYGALFTAFQALVDEGDEVIIIEPFFDCYEPMTMMAGGRPVFVSLKPGPIQNGELGSSSNWQLDPMELAGKFTSRTKALVLNTPNNPLGKVFSREELELVASLCQQHDVVCITDEVYQWMVYDGHQHISIASLPGMWERTLTIGSAGKTFSATGWKVGWVLGPDHIMKHLRTVHQNSVFHCPTQSQAAVAESFEREQLLFRQPSSYFVQFPQAMQRCRDHMIRSLQSVGLKPIIPQGSYFLITDISDFKRKMPDLPGAVDEPYDRRFVKWMIKNKGLVAIPVSIFYSVPHQKHFDHYIRFCFVKDEATLQAMDEKLRKWKVEL

SEQ ID NO: 2 - protein, 422 aa, Homo sapiens
MAKQLQARRLDGIDYNPWVEFVKLASEHDVVNLGQGFPDFPPPDFAVEAFQHAVSGDFMLNQYTKTFGYPPLTKILASFFGELLGQEIDPLRNVLVTVGGHGALFTAFQALVDEGDEVIIIEPFFDCYEPMTMMAGGRPVFVSLKPGPIQNGELGSSSNWQLDPMELAGKFTSRTKALVLNTPNNPLGKVFSREELELVASLCQQHDVVCITDEVYQWMVYDGHQHISIASLPGMWERTLTIGSAGKTFSATGWKVGWVLGPDHIMKHLRTVHQNSVFHCPTQSQAAVAESFEREQLLFRQPSSYFVQFPQAMQRCRDHMIRSLQSVGLKPIIPQGSYFLITDISDFKRKMPDLPGAVDEPYDRRFVKWMIKNKGLVAIPVSIFYSVPHQKHFDHYIRFCFVKDEATLQAMDEKLRKWKVEL

SEQ ID NO: 3 - protein, 422 aa, Homo sapiens
MAKQLQARRLDGIDYNPWVEFVKLASEHDVVNLGQGFPDFPPPDFAVEAFQHAVSGDFMLNQYTKTFGYPPLTKILASFFGELLGQEIDPLRNVLVTVGGYGALFTAFQALVDEGDEVIIIEPFFDCYEPMTMMAGGRPVFVSLKPGPIQNGELGSSSNWQLDPMELAGKFTSRTKALVLNTPNNPLGKVFSREELELVASLCQQHDVVCITDEVYQWMVYDGHQHISIASLPGMWERTLTIGSAGKTFSATGWKVGWVLGPDHIMKHLRTVHQNSVFFCPTQSQAAVAESFEREQLLFRQPSSYFVQFPQAMQRCRDHMIRSLQSVGLKPIIPQGSYFLITDISDFKRKMPDLPGAVDEPYDRRFVKWMIKNKGLVAIPVSIFYSVPHQKHFDHYIRFCFVKDEATLQAMDEKLRKWKVEL